European Patent Specification EP 3 858 868 B1, published October 22, 2025. Title: POLYPEPTIDE COMPOSITION. Applicant: SHANGHAI JIAOTONG UNIVERSITY JECHO LABORATORIES, INC. Application WO2019CN108588. The sequence listing filed with the application follows.

SEQUENCE LISTING (16 sequences)

SEQ ID NO: 1 - protein, 344 aa, Artificial Sequence
  Truncated form PE38
GGSLAALTAHQACHLPLETFTRHRQPRGWEQLEQCGYPVQRLVALYLAARLSWNQVDQVIRNALASPGSGGDLGEAIREQPEQARLALTLAAAESERFVRQGTGNDEAGAASGPADSGDALLERNYPTGAEFLGDGGDISFSTRGTQNWTVERLLQAHRQLEERGYVFVGYHGTFLEAAQSIVFGGVRARSQDLDAIWRGFYIAGDPALAYGYAQDQEPDARGRIRNGALLRVYVPRSSLPGFYRTGLTLAAPEAAGEVERLIGHPLPLRLDAITGPEEEGGRLETILGWPLAERTVVIPSAIPTDPRNVGGDLDPSSIPDKEQAISALPDYASQPGKPPKDEL

SEQ ID NO: 2 - protein, 102 aa, Artificial Sequence
  First intein fragment
CLSYETEILTVEYGLLPIGKIVEKRIECTVYSVDNNGNIYTQPVAQWHDRGEQEVFEYCLEDGSLIRATKDHKFMTVDGQMLPIDEIFERELDLMRVDNLPN

SEQ ID NO: 3 - protein, 36 aa, Artificial Sequence
  Second intein fragment
MIKIATRKYLGKQNVYDIGVERDHNFALKNGFIASN

SEQ ID NO: 4 - protein, 139 aa, Artificial Sequence
  First toxin fragment
GGSLAALTAHQACHLPLETFTRHRQPRGWEQLEQCGYPVQRLVALYLAARLSWNQVDQVIRNALASPGSGGDLGEAIREQPEQARLALTLAAAESERFVRQGTGNDEAGAASGPADSGDALLERNYPTGAEFLGDGGDI

SEQ ID NO: 5 - protein, 205 aa, Artificial Sequence
  Second toxin fragment
SFSTRGTQNWTVERLLQAHRQLEERGYVFVGYHGTFLEAAQSIVFGGVRARSQDLDAIWRGFYIAGDPALAYGYAQDQEPDARGRIRNGALLRVYVPRSSLPGFYRTGLTLAAPEAAGEVERLIGHPLPLRLDAITGPEEEGGRLETILGWPLAERTVVIPSAIPTDPRNVGGDLDPSSIPDKEQAISALPDYASQPGKPPKDEL

SEQ ID NO: 6 - protein, 484 aa, Artificial Sequence
  First polypeptide comprising targeting portion
MDIQMTQSPSSLSASVGDRVTITCRASQDVNTAVAWYQQKPGKAPKLLIYSASFLYSGVPSRFSGSRSGTDFTLTISSLQPEDFATYYCQQHYTTPPTFGQGTKVEIKGGGGSGGGGSGGGGSEVQLVESGGGLVQPGGSLRLSCAASGFNIKDTYIHWVRQAPGKGLEWVARIYPTNGYTRYADSVKGRFTISADTSKNTAYLQMNSLRAEDTAVYYCSRWGGDGFYAMDYWGQGTLVTVSSGGSLAALTAHQACHLPLETFTRHRQPRGWEQLEQCGYPVQRLVALYLAARLSWNQVDQVIRNALASPGSGGDLGEAIREQPEQARLALTLAAAESERFVRQGTGNDEAGAASGPADSGDALLERNYPTGAEFLGDGGDICLSYETEILTVEYGLLPIGKIVEKRIECTVYSVDNNGNIYTQPVAQWHDRGEQEVFEYCLEDGSLIRATKDHKFMTVDGQMLPIDEIFERELDLMRVDNLPN

SEQ ID NO: 7 - protein, 484 aa, Artificial Sequence
  Second polypeptide comprising targeting portion
MDIQMTQSPSSLSASVGDRVTITCRASQDVNTAVAWYQQKPGKAPKLLIYSASFLYSGVPSRFSGSRSGTDFTLTISSLQPEDFATYYCQQHYTTPPTFGQGTKVEIKGGGGSGGGGSGGGGSEVQLVESGGGLVQPGGSLRLSCAASGFNIKDTYIHWVRQAPGKGLEWVARIYPTNGYTRYADSVKGRFTISADTSKNTAYLQMNSLRAEDTAVYYCSRWGGDGFYAMDYWGQGTLVTVSSMIKIATRKYLGKQNVYDIGVERDHNFALKNGFIASNCFNTRGTQNWTVERLLQAHRQLEERGYVFVGYHGTFLEAAQSIVFGGVRARSQDLDAIWRGFYIAGDPALAYGYAQDQEPDARGRIRNGALLRVYVPRSSLPGFYRTGLTLAAPEAAGEVERLIGHPLPLRLDAITGPEEEGGRLETILGWPLAERTVVIPSAIPTDPRNVGGDLDPSSIPDKEQAISALPDYASQPGKPPKDEL

SEQ ID NO: 8 - protein, 243 aa, Artificial Sequence
  Targeting portion scFv
MDIQMTQSPSSLSASVGDRVTITCRASQDVNTAVAWYQQKPGKAPKLLIYSASFLYSGVPSRFSGSRSGTDFTLTISSLQPEDFATYYCQQHYTTPPTFGQGTKVEIKGGGGSGGGGSGGGGSEVQLVESGGGLVQPGGSLRLSCAASGFNIKDTYIHWVRQAPGKGLEWVARIYPTNGYTRYADSVKGRFTISADTSKNTAYLQMNSLRAEDTAVYYCSRWGGDGFYAMDYWGQGTLVTVSS

SEQ ID NO: 9 - protein, 587 aa, Artificial Sequence
  scFvPE38
MDIQMTQSPSSLSASVGDRVTITCRASQDVNTAVAWYQQKPGKAPKLLIYSASFLYSGVPSRFSGSRSGTDFTLTISSLQPEDFATYYCQQHYTTPPTFGQGTKVEIKGGGGSGGGGSGGGGSEVQLVESGGGLVQPGGSLRLSCAASGFNIKDTYIHWVRQAPGKGLEWVARIYPTNGYTRYADSVKGRFTISADTSKNTAYLQMNSLRAEDTAVYYCSRWGGDGFYAMDYWGQGTLVTVSSGGSLAALTAHQACHLPLETFTRHRQPRGWEQLEQCGYPVQRLVALYLAARLSWNQVDQVIRNALASPGSGGDLGEAIREQPEQARLALTLAAAESERFVRQGTGNDEAGAASGPADSGDALLERNYPTGAEFLGDGGDISFSTRGTQNWTVERLLQAHRQLEERGYVFVGYHGTFLEAAQSIVFGGVRARSQDLDAIWRGFYIAGDPALAYGYAQDQEPDARGRIRNGALLRVYVPRSSLPGFYRTGLTLAAPEAAGEVERLIGHPLPLRLDAITGPEEEGGRLETILGWPLAERTVVIPSAIPTDPRNVGGDLDPSSIPDKEQAISALPDYASQPGKPPKDEL

SEQ ID NO: 10 - protein, 587 aa, Artificial Sequence
  scFvPM1
MDIQMTQSPSSLSASVGDRVTITCRASQDVNTAVAWYQQKPGKAPKLLIYSASFLYSGVPSRFSGSRSGTDFTLTISSLQPEDFATYYCQQHYTTPPTFGQGTKVEIKGGGGSGGGGSGGGGSEVQLVESGGGLVQPGGSLRLSCAASGFNIKDTYIHWVRQAPGKGLEWVARIYPTNGYTRYADSVKGRFTISADTSKNTAYLQMNSLRAEDTAVYYCSRWGGDGFYAMDYWGQGTLVTVSSGGSLAALTAHQACHLPLETFTRHRQPRGWEQLEQCGYPVQRLVALYLAARLSWNQVDQVIRNALASPGSGGDLGEAIREQPEQARLALTLAAAESERFVRQGTGNDEAGAASGPADSGDALLERNYPTGAEFLGDGGDICFNTRGTQNWTVERLLQAHRQLEERGYVFVGYHGTFLEAAQSIVFGGVRARSQDLDAIWRGFYIAGDPALAYGYAQDQEPDARGRIRNGALLRVYVPRSSLPGFYRTGLTLAAPEAAGEVERLIGHPLPLRLDAITGPEEEGGRLETILGWPLAERTVVIPSAIPTDPRNVGGDLDPSSIPDKEQAISALPDYASQPGKPPKDEL

SEQ ID NO: 11 - protein, 587 aa, Artificial Sequence
  scFvPM2
MDIQMTQSPSSLSASVGDRVTITCRASQDVNTAVAWYQQKPGKAPKLLIYSASFLYSGVPSRFSGSRSGTDFTLTISSLQPEDFATYYCQQHYTTPPTFGQGTKVEIKGGGGSGGGGSGGGGSEVQLVESGGGLVQPGGSLRLSCAASGFNIKDTYIHWVRQAPGKGLEWVARIYPTNGYTRYADSVKGRFTISADTSKNTAYLQMNSLRAEDTAVYYCSRWGGDGFYAMDYWGQGTLVTVSSGGSLAALTAHQACHLPLETFTRHRQPRGWEQLEQCGYPVQRLVALYLAARLSWNQVDQVIRNALASPGSGGDLGEAIREQPEQARLALTLAAAESERFVRQGTGNDEAGAASGPADSGDALLERNYPTGAEFLGDGGDISFSTRGTQNWTVERLLQAHRQLEERGYVFVGYHGTFLEAAQSIVFGGVRARSQDLDAIWRGFYIAGDPALAYGYAQDQEPCFNGRIRNGALLRVYVPRSSLPGFYRTGLTLAAPEAAGEVERLIGHPLPLRLDAITGPEEEGGRLETILGWPLAERTVVIPSAIPTDPRNVGGDLDPSSIPDKEQAISALPDYASQPGKPPKDEL

SEQ ID NO: 12 - protein, 587 aa, Artificial Sequence
  scFvPM3
MDIQMTQSPSSLSASVGDRVTITCRASQDVNTAVAWYQQKPGKAPKLLIYSASFLYSGVPSRFSGSRSGTDFTLTISSLQPEDFATYYCQQHYTTPPTFGQGTKVEIKGGGGSGGGGSGGGGSEVQLVESGGGLVQPGGSLRLSCAASGFNIKDTYIHWVRQAPGKGLEWVARIYPTNGYTRYADSVKGRFTISADTSKNTAYLQMNSLRAEDTAVYYCSRWGGDGFYAMDYWGQGTLVTVSSGGSLAALTAHQACHLPLETFTRHRQPRGWEQLEQCGYPVQRLVALYLAARLSWNQVDQVIRNALASPGSGGDLGEAIREQPEQARLALTLAAAESERFVRQGTGNDEAGAASGPADSGDALLERNYPTGAEFLGDGGDISFSTRGTQNWTVERLLQAHRQLEERGYVFVGYHGTFLEAAQSIVFGGVRARSQDLDAIWRGFYIAGDPALAYGYAQDQEPDARGRIRNGALLRVYVPRSSLPGFYRTGLTLAAPEAAGEVERLIGHPLCFNLDAITGPEEEGGRLETILGWPLAERTVVIPSAIPTDPRNVGGDLDPSSIPDKEQAISALPDYASQPGKPPKDEL

SEQ ID NO: 13 - protein, 382 aa, Artificial Sequence
  scFvPn
MDIQMTQSPSSLSASVGDRVTITCRASQDVNTAVAWYQQKPGKAPKLLIYSASFLYSGVPSRFSGSRSGTDFTLTISSLQPEDFATYYCQQHYTTPPTFGQGTKVEIKGGGGSGGGGSGGGGSEVQLVESGGGLVQPGGSLRLSCAASGFNIKDTYIHWVRQAPGKGLEWVARIYPTNGYTRYADSVKGRFTISADTSKNTAYLQMNSLRAEDTAVYYCSRWGGDGFYAMDYWGQGTLVTVSSGGSLAALTAHQACHLPLETFTRHRQPRGWEQLEQCGYPVQRLVALYLAARLSWNQVDQVIRNALASPGSGGDLGEAIREQPEQARLALTLAAAESERFVRQGTGNDEAGAASGPADSGDALLERNYPTGAEFLGDGGDI

SEQ ID NO: 14 - protein, 205 aa, Artificial Sequence
  Pc
CFNTRGTQNWTVERLLQAHRQLEERGYVFVGYHGTFLEAAQSIVFGGVRARSQDLDAIWRGFYIAGDPALAYGYAQDQEPDARGRIRNGALLRVYVPRSSLPGFYRTGLTLAAPEAAGEVERLIGHPLPLRLDAITGPEEEGGRLETILGWPLAERTVVIPSAIPTDPRNVGGDLDPSSIPDKEQAISALPDYASQPGKPPKDEL

SEQ ID NO: 15 - protein, 241 aa, Artificial Sequence
  Second polypeptide not comprising targeting portion (IcPc)
MIKIATRKYLGKQNVYDIGVERDHNFALKNGFIASNCFNTRGTQNWTVERLLQAHRQLEERGYVFVGYHGTFLEAAQSIVFGGVRARSQDLDAIWRGFYIAGDPALAYGYAQDQEPDARGRIRNGALLRVYVPRSSLPGFYRTGLTLAAPEAAGEVERLIGHPLPLRLDAITGPEEEGGRLETILGWPLAERTVVIPSAIPTDPRNVGGDLDPSSIPDKEQAISALPDYASQPGKPPKDEL

SEQ ID NO: 16 - protein, 344 aa, Artificial Sequence
  Truncated form PM1
GGSLAALTAHQACHLPLETFTRHRQPRGWEQLEQCGYPVQRLVALYLAARLSWNQVDQVIRNALASPGSGGDLGEAIREQPEQARLALTLAAAESERFVRQGTGNDEAGAASGPADSGDALLERNYPTGAEFLGDGGDICFNTRGTQNWTVERLLQAHRQLEERGYVFVGYHGTFLEAAQSIVFGGVRARSQDLDAIWRGFYIAGDPALAYGYAQDQEPDARGRIRNGALLRVYVPRSSLPGFYRTGLTLAAPEAAGEVERLIGHPLPLRLDAITGPEEEGGRLETILGWPLAERTVVIPSAIPTDPRNVGGDLDPSSIPDKEQAISALPDYASQPGKPPKDEL